European Patent Application EP 4 410 978 A2, published August 7, 2024. Title: METHODS FOR QUANTITATIVE GENETIC ANALYSIS OF CELL FREE DNA. Applicant: Resolution Bioscience, Inc. Application EP PCT/US2014/052317, filed August 22, 2014. The sequence listing filed with the application follows.

SEQUENCE LISTING (562 sequences)

SEQ ID NO: 1 - DNA, 60 bp, synthetic construct
  misc_feature 1..60: note = Probe
  source 1..60: mol_type = other DNA
taaacattggaaaggtttctaattaaccaggagatccaaaagaaagcggttcaagtagca

SEQ ID NO: 2 - DNA, 60 bp, synthetic construct
  misc_feature 1..60: note = Probe
  source 1..60: mol_type = other DNA
gatctcagtttttttggttaactatgtattttggtatatgaagcttctgggttttgcaca

SEQ ID NO: 3 - DNA, 60 bp, synthetic construct
  misc_feature 1..60: note = Probe
  source 1..60: mol_type = other DNA
gacagataagcatacatattaacatggatatatatgtgaatttcattcaaatggttctca

SEQ ID NO: 4 - DNA, 60 bp, synthetic construct
  misc_feature 1..60: note = Probe
  source 1..60: mol_type = other DNA
agctcttagcctttggggggatgacactcttgagcggacgtggggacgcctcgctcttta

SEQ ID NO: 5 - DNA, 60 bp, synthetic construct
  misc_feature 1..60: note = Probe
  source 1..60: mol_type = other DNA
aagcccccaccgccgcctctttccaaaataaacaccagccagccgccgagcccggagtcg

SEQ ID NO: 6 - DNA, 60 bp, synthetic construct
  misc_feature 1..60: note = Probe
  source 1..60: mol_type = other DNA
gcctcccttccccctccccgcccgacagcggccgctcgggccccggctctcggttataag

SEQ ID NO: 7 - DNA, 60 bp, synthetic construct
  misc_feature 1..60: note = Probe
  source 1..60: mol_type = other DNA
ggtgtggcagccaggggggcgcactctgctctggctgggccccttctcccatgttttctt

SEQ ID NO: 8 - DNA, 60 bp, synthetic construct
  misc_feature 1..60: note = Probe
  source 1..60: mol_type = other DNA
ttacacaacctttgggcttggacaacactttggggtccaaagaacctaagagtctttctg

SEQ ID NO: 9 - DNA, 60 bp, synthetic construct
  misc_feature 1..60: note = Probe
  source 1..60: mol_type = other DNA
tgatgaaacttgggctggatggggcacaggtagggtgcttgttgctttcagtcagatgaa

SEQ ID NO: 10 - DNA, 60 bp, synthetic construct
  misc_feature 1..60: note = Probe
  source 1..60: mol_type = other DNA
aatgaaagaaaaggaggccagattgctactcctggtccctgccacacactaggtacccta

SEQ ID NO: 11 - DNA, 60 bp, synthetic construct
  misc_feature 1..60: note = Probe
  source 1..60: mol_type = other DNA
attgacaatacctacataaaactctttccagaatgttgttaagtcttagtcattagggag

SEQ ID NO: 12 - DNA, 60 bp, synthetic construct
  misc_feature 1..60: note = Probe
  source 1..60: mol_type = other DNA
ggatttccaccaacactgtattcatgtacccatttttctcttaacctaactttattggtc

SEQ ID NO: 13 - DNA, 60 bp, synthetic construct
  misc_feature 1..60: note = Probe
  source 1..60: mol_type = other DNA
caaagggggaaaaccatcaggacattatttaacaacggaaatatctaactgaaaggcaaa

SEQ ID NO: 14 - DNA, 60 bp, synthetic construct
  misc_feature 1..60: note = Probe
  source 1..60: mol_type = other DNA
caggcagaccaaccaaagtctttgttccaccttttaaaactaaatcacattttcacagag

SEQ ID NO: 15 - DNA, 60 bp, synthetic construct
  misc_feature 1..60: note = Probe
  source 1..60: mol_type = other DNA
ccccagccagcggtccgcaacccttgccgcatccacgaaactttgcccatagcagcgggc

SEQ ID NO: 16 - DNA, 60 bp, synthetic construct
  misc_feature 1..60: note = Probe
  source 1..60: mol_type = other DNA
cgactcatctcagcattaaagtgataaaaaaataaattaaaaggcaagtggacttcggtg

SEQ ID NO: 17 - DNA, 60 bp, synthetic construct
  misc_feature 1..60: note = Probe
  source 1..60: mol_type = other DNA
ctgtggcgcgcactgcgcgctgcgccaggtttccgcaccaagacccctttaactcaagac

SEQ ID NO: 18 - DNA, 60 bp, synthetic construct
  misc_feature 1..60: note = Probe
  source 1..60: mol_type = other DNA
ttctactgcgacgaggaggagaacttctaccagcagcagcagcagagcgagctgcagccc

SEQ ID NO: 19 - DNA, 60 bp, synthetic construct
  misc_feature 1..60: note = Probe
  source 1..60: mol_type = other DNA
accgagctgctgggaggagacatggtgaaccagagtttcatctgcgacccggacgacgag

SEQ ID NO: 20 - DNA, 60 bp, synthetic construct
  misc_feature 1..60: note = Probe
  source 1..60: mol_type = other DNA
gccgccgcctcagagtgcatcgacccctcggtggtcttcccctaccctctcaacgacagc

SEQ ID NO: 21 - DNA, 60 bp, synthetic construct
  misc_feature 1..60: note = Probe
  source 1..60: mol_type = other DNA
ggcggctaggggacaggggcggggtgggcagcagctcgaatttcttccagatatcctcgc

SEQ ID NO: 22 - DNA, 60 bp, synthetic construct
  misc_feature 1..60: note = Probe
  source 1..60: mol_type = other DNA
agacgagcttggcggcggccgagaagccgctccacatacagtcctggatgatgatgtttt

SEQ ID NO: 23 - DNA, 60 bp, synthetic construct
  misc_feature 1..60: note = Probe
  source 1..60: mol_type = other DNA
aggagagcagagaatccgaggacggagagaaggcgctggagtcttgcgaggcgcaggact

SEQ ID NO: 24 - DNA, 60 bp, synthetic construct
  misc_feature 1..60: note = Probe
  source 1..60: mol_type = other DNA
taagagtggcccgttaaataagctgccaatgaaaatgggaaaggtatccagccgcccact

SEQ ID NO: 25 - DNA, 60 bp, synthetic construct
  misc_feature 1..60: note = Probe
  source 1..60: mol_type = other DNA
ttgtatttgtacagcattaatctggtaattgattattttaatgtaaccttgctaaaggag

SEQ ID NO: 26 - DNA, 60 bp, synthetic construct
  misc_feature 1..60: note = Probe
  source 1..60: mol_type = other DNA
gaggccacagcaaacctcctcacagcccactggtcctcaagaggtgccacgtctccacac

SEQ ID NO: 27 - DNA, 60 bp, synthetic construct
  misc_feature 1..60: note = Probe
  source 1..60: mol_type = other DNA
agaggaggaacgagctaaaacggagcttttttgccctgcgtgaccagatcccggagttgg

SEQ ID NO: 28 - DNA, 60 bp, synthetic construct
  misc_feature 1..60: note = Probe
  source 1..60: mol_type = other DNA
tccaacttgaccctcttggcagcaggatagtccttccgagtggagggaggcgctgcgtag

SEQ ID NO: 29 - DNA, 60 bp, synthetic construct
  misc_feature 1..60: note = Probe
  source 1..60: mol_type = other DNA
gcttggacggacaggatgtatgctgtggcttttttaaggataactaccttgggggccttt

SEQ ID NO: 30 - DNA, 60 bp, synthetic construct
  misc_feature 1..60: note = Probe
  source 1..60: mol_type = other DNA
gcatttgatcatgcatttgaaacaagttcataggtgattgctcaggacatttctgttaga

SEQ ID NO: 31 - DNA, 60 bp, synthetic construct
  misc_feature 1..60: note = Probe
  source 1..60: mol_type = other DNA
cgccccgcgccctcccagccgggtccagccggagccatggggccggagccgcagtgagca

SEQ ID NO: 32 - DNA, 60 bp, synthetic construct
  misc_feature 1..60: note = Probe
  source 1..60: mol_type = other DNA
ctctggccccgccggccgcgggacctcggcggggcatccacagggcagggtcccgccgct

SEQ ID NO: 33 - DNA, 60 bp, synthetic construct
  misc_feature 1..60: note = Probe
  source 1..60: mol_type = other DNA
ggcatgacttggagtgagtttggatggggtggccaggtctgagaaggtcccccgccagtg

SEQ ID NO: 34 - DNA, 60 bp, synthetic construct
  misc_feature 1..60: note = Probe
  source 1..60: mol_type = other DNA
gcagggcaccttcttctgccacccacctgtaaacagagggctcagcccagctggaggcag

SEQ ID NO: 35 - DNA, 60 bp, synthetic construct
  misc_feature 1..60: note = Probe
  source 1..60: mol_type = other DNA
cccaagatctccaagtactggggaaccccagggaggccctggggggtggcagtgttccta

SEQ ID NO: 36 - DNA, 60 bp, synthetic construct
  misc_feature 1..60: note = Probe
  source 1..60: mol_type = other DNA
ctaatgcacacaaagcctccccctggttagcagtggccctggtcagctctgaataaccaa

SEQ ID NO: 37 - DNA, 60 bp, synthetic construct
  misc_feature 1..60: note = Probe
  source 1..60: mol_type = other DNA
ctgctcctcttttagaaggcaggagggccccaagggaagcagaaggtgacagaaggggaa

SEQ ID NO: 38 - DNA, 60 bp, synthetic construct
  misc_feature 1..60: note = Probe
  source 1..60: mol_type = other DNA
tggggcagtggcgggcaggcactgggttgtaagttgggagtttgcggctggggtcaggct

SEQ ID NO: 39 - DNA, 60 bp, synthetic construct
  misc_feature 1..60: note = Probe
  source 1..60: mol_type = other DNA
tctgctgctgtttgtgcctctctctgttactaacccgtcctctcgctgttagacatctct

SEQ ID NO: 40 - DNA, 60 bp, synthetic construct
  misc_feature 1..60: note = Probe
  source 1..60: mol_type = other DNA
cccacccctcccatgtcacctgtatgacacctgcattccacccggccccagccctcccct

SEQ ID NO: 41 - DNA, 60 bp, synthetic construct
  misc_feature 1..60: note = Probe
  source 1..60: mol_type = other DNA
tgggccaggtagtctccctagaaggtgatgctgatgagggtctggtgcccagggcgccac

SEQ ID NO: 42 - DNA, 60 bp, synthetic construct
  misc_feature 1..60: note = Probe
  source 1..60: mol_type = other DNA
ggtgcccaccccttgcatcctggggggtagagcacattgggcacaaagcagaggcacata

SEQ ID NO: 43 - DNA, 60 bp, synthetic construct
  misc_feature 1..60: note = Probe
  source 1..60: mol_type = other DNA
caccctgcctggtactgccctattgcccctggcacaccagggcaaaacagcacagtgaaa

SEQ ID NO: 44 - DNA, 60 bp, synthetic construct
  misc_feature 1..60: note = Probe
  source 1..60: mol_type = other DNA
ccatttacagaaacaaacctccccaccaaaatgagaaaactgtgtttctccctggcactc

SEQ ID NO: 45 - DNA, 60 bp, synthetic construct
  misc_feature 1..60: note = Probe
  source 1..60: mol_type = other DNA
ttattcttcttgtgcctgggcacggtaatgctgctcatggtggtgcacgaagggccaggg

SEQ ID NO: 46 - DNA, 60 bp, synthetic construct
  misc_feature 1..60: note = Probe
  source 1..60: mol_type = other DNA
gaaggataggacagggtgggctgggccaggctgcatgcgcagagggacaggaactgcagc

SEQ ID NO: 47 - DNA, 60 bp, synthetic construct
  misc_feature 1..60: note = Probe
  source 1..60: mol_type = other DNA
gggcccggaccctgatgctcatgtggctgttgacctgtcccggtatgaaggctgagacgg

SEQ ID NO: 48 - DNA, 60 bp, synthetic construct
  misc_feature 1..60: note = Probe
  source 1..60: mol_type = other DNA
tctgtctcctgccatccccaagagatgctgccacatctggatcctcaggactctgtctgc

SEQ ID NO: 49 - DNA, 60 bp, synthetic construct
  misc_feature 1..60: note = Probe
  source 1..60: mol_type = other DNA
tcacgtcccagggcagttttcttccctgaagaaagttggatggcatgatctgtcttccca

SEQ ID NO: 50 - DNA, 60 bp, synthetic construct
  misc_feature 1..60: note = Probe
  source 1..60: mol_type = other DNA
gtgttgagaacagactactgacttctaatagcagcgacttctttaccttgataaaccaca

SEQ ID NO: 51 - DNA, 60 bp, synthetic construct
  misc_feature 1..60: note = Probe
  source 1..60: mol_type = other DNA
aaaaaaaggatgggttccatatgggtggtgtcaagtgcccacctcctagcaagtcagcag

SEQ ID NO: 52 - DNA, 60 bp, synthetic construct
  misc_feature 1..60: note = Probe
  source 1..60: mol_type = other DNA
ccctcacaaggtcaaagctatacatcagctcctgtgacattgactcatcccccagacctt

SEQ ID NO: 53 - DNA, 60 bp, synthetic construct
  misc_feature 1..60: note = Probe
  source 1..60: mol_type = other DNA
aacccaccgagatctgcaaactttgcaggatgcaccagatgtcttgtagccatgggtcaa

SEQ ID NO: 54 - DNA, 60 bp, synthetic construct
  misc_feature 1..60: note = TYMSr4r probe
  source 1..60: mol_type = other DNA
tgcctccctcaggtgcctctgcacaaaaccagattgcttccctctaagagtatggttagt

SEQ ID NO: 55 - DNA, 60 bp, synthetic construct
  misc_feature 1..60: note = Probe
  source 1..60: mol_type = other DNA
gttttactttgcctttagctgtggtctttcaaaccaccatccctccttatcttcctctgc

SEQ ID NO: 56 - DNA, 60 bp, synthetic construct
  misc_feature 1..60: note = Probe
  source 1..60: mol_type = other DNA
ctctgcaatttgttttcccatattaaagaactgaagagctcagtgtggtaggctggcaag

SEQ ID NO: 57 - DNA, 60 bp, synthetic construct
  misc_feature 1..60: note = Probe
  source 1..60: mol_type = other DNA
ttttaaatgatgttttaaagaattgaaactaacatactgttctgctttctcccccgggtt

SEQ ID NO: 58 - DNA, 60 bp, synthetic construct
  misc_feature 1..60: note = Probe
  source 1..60: mol_type = other DNA
cctgcccaccacttctccctaaactgaagccccacatttggagcagtcatctttatcttg

SEQ ID NO: 59 - DNA, 60 bp, synthetic construct
  misc_feature 1..60: note = Probe
  source 1..60: mol_type = other DNA
ggttgcgctccaatcatgttacataacctacggcaaggtatcgacaggatcatactcctg

SEQ ID NO: 60 - DNA, 60 bp, synthetic construct
  misc_feature 1..60: note = Probe
  source 1..60: mol_type = other DNA
gcacagttacatttgccagtggcaacatccttaaaaattaataactgataggtcacggac

SEQ ID NO: 61 - DNA, 60 bp, synthetic construct
  misc_feature 1..60: note = Probe
  source 1..60: mol_type = other DNA
cgtcccgccgcgccacttggcctgcctccgtcccgccgcgccacttcgcctgcctccgtc

SEQ ID NO: 62 - DNA, 60 bp, synthetic construct
  misc_feature 1..60: note = Probe
  source 1..60: mol_type = other DNA
ctgtaaggcgaggaggacgatgcgtcccctccctcgcaggattgaggttaggactaaacg

SEQ ID NO: 63 - DNA, 35 bp, synthetic construct
  misc_feature 1..35: note = Partner Oligo #138
  source 1..35: mol_type = other DNA
gtgaaaaccaggatcaactcccgtgccagtcacat

SEQ ID NO: 64 - DNA, 20 bp, synthetic construct
  misc_feature 1..20: note = Adaptor
  misc_feature 1..8: note = n is a, c, g, or t
  source 1..20: mol_type = other DNA
nnnnnnnncatggccgcagg

SEQ ID NO: 65 - DNA, 20 bp, synthetic construct
  misc_feature 1..20: note = Adaptor
  misc_feature 1..8: note = n is a, c, g, or t
  source 1..20: mol_type = other DNA
nnnnnnnnatcttagtggca

SEQ ID NO: 66 - DNA, 20 bp, synthetic construct
  misc_feature 1..20: note = Adaptor
  misc_feature 1..8: note = n is a, c, g, or t
  source 1..20: mol_type = other DNA
nnnnnnnncggaactcggag

SEQ ID NO: 67 - DNA, 20 bp, synthetic construct
  misc_feature 1..20: note = Adaptor
  misc_feature 1..8: note = n is a, c, g, or t
  source 1..20: mol_type = other DNA
nnnnnnnngactccgatccc

SEQ ID NO: 68 - DNA, 95 bp, synthetic construct
  misc_feature 1..95: note = Probe
  source 1..95: mol_type = other DNA
atgtgactggcacgggagttgatcctggttttcacgggtttgagtggcatgagctacctactggatgtgcctgactgtttccccttcttcttccc

SEQ ID NO: 69 - DNA, 95 bp, synthetic construct
  misc_feature 1..95: note = Probe
  source 1..95: mol_type = other DNA
atgtgactggcacgggagttgatcctggttttcacctatctccaggatggagagagggaaaaaaaagatgggtctgtgtgggagggcaggtactt

SEQ ID NO: 70 - DNA, 95 bp, synthetic construct
  misc_feature 1..95: note = Probe
  source 1..95: mol_type = other DNA
atgtgactggcacgggagttgatcctggttttcacgaaagaagccaggtcttcaattaataagattccctggtctcgtttgtctacctgttaatg

SEQ ID NO: 71 - DNA, 95 bp, synthetic construct
  misc_feature 1..95: note = Probe
  source 1..95: mol_type = other DNA
atgtgactggcacgggagttgatcctggttttcaccagactcgcgcccaattttcccccaccccttgttattgccacaaaatcctgaggatgatc

SEQ ID NO: 72 - DNA, 95 bp, synthetic construct
  misc_feature 1..95: note = Probe
  source 1..95: mol_type = other DNA
atgtgactggcacgggagttgatcctggttttcacaagcacctagccccattcctgctgagcaggaggtggcaggtaccccagactgggaggtaa

SEQ ID NO: 73 - DNA, 95 bp, synthetic construct
  misc_feature 1..95: note = Probe
  source 1..95: mol_type = other DNA
atgtgactggcacgggagttgatcctggttttcacagtcggtggggccaggatgaggcccagtctgttcacacatggctgctgcctctcagctct

SEQ ID NO: 74 - DNA, 95 bp, synthetic construct
  misc_feature 1..95: note = Probe
  source 1..95: mol_type = other DNA
atgtgactggcacgggagttgatcctggttttcaccctggccctcagccagtacagaaagtcatttgtcaaggccttcagttggcagacgtgctc

SEQ ID NO: 75 - DNA, 95 bp, synthetic construct
  misc_feature 1..95: note = Probe
  source 1..95: mol_type = other DNA
atgtgactggcacgggagttgatcctggttttcacagaattcattgccagctataaatctgtggaaacgctgccacacaatcttagcacacaaga

SEQ ID NO: 76 - DNA, 95 bp, synthetic construct
  misc_feature 1..95: note = Probe
  source 1..95: mol_type = other DNA
atgtgactggcacgggagttgatcctggttttcacttacttccctccagttttgttgcttgcaaaacaacagaatcttctctccatgaaatcatg

SEQ ID NO: 77 - DNA, 95 bp, synthetic construct
  misc_feature 1..95: note = Probe
  source 1..95: mol_type = other DNA
atgtgactggcacgggagttgatcctggttttcaccaggggtatctattatccccattttctcacaaaggaaaccaagataaaaggtttaaatgg

SEQ ID NO: 78 - DNA, 95 bp, synthetic construct
  misc_feature 1..95: note = Probe
  source 1..95: mol_type = other DNA
atgtgactggcacgggagttgatcctggttttcactgttacctttaaaagacatctgctttctgccaaaattaatgtgctgaacttaaacttacc

SEQ ID NO: 79 - DNA, 95 bp, synthetic construct
  misc_feature 1..95: note = Probe
  source 1..95: mol_type = other DNA
atgtgactggcacgggagttgatcctggttttcacttcccagtaaattactcttaccaatgcaacagactttaaagaagttgtgttttacaatgc

SEQ ID NO: 80 - DNA, 95 bp, synthetic construct
  misc_feature 1..95: note = Probe
  source 1..95: mol_type = other DNA
atgtgactggcacgggagttgatcctggttttcactaaatgacataacagttatgattttgcagaaaacagatctgtatttatttcagtgttact

SEQ ID NO: 81 - DNA, 95 bp, synthetic construct
  misc_feature 1..95: note = Probe
  source 1..95: mol_type = other DNA
atgtgactggcacgggagttgatcctggttttcacgacaggttttgaaagatatttgtgttactaatgactgtgctataacttttttttctttcc

SEQ ID NO: 82 - DNA, 95 bp, synthetic construct
  misc_feature 1..95: note = Probe
  source 1..95: mol_type = other DNA
atgtgactggcacgggagttgatcctggttttcacctgtggcgcgcactgcgcgctgcgccaggtttccgcaccaagacccctttaactcaagac

SEQ ID NO: 83 - DNA, 95 bp, synthetic construct
  misc_feature 1..95: note = Probe
  source 1..95: mol_type = other DNA
atgtgactggcacgggagttgatcctggttttcacggcggctaggggacaggggcggggtgggcagcagctcgaatttcttccagatatcctcgc

SEQ ID NO: 84 - DNA, 95 bp, synthetic construct
  misc_feature 1..95: note = Probe
  source 1..95: mol_type = other DNA
atgtgactggcacgggagttgatcctggttttcacaccgagctgctgggaggagacatggtgaaccagagtttcatctgcgacccggacgacgag

SEQ ID NO: 85 - DNA, 95 bp, synthetic construct
  misc_feature 1..95: note = Probe
  source 1..95: mol_type = other DNA
atgtgactggcacgggagttgatcctggttttcacaggagagcagagaatccgaggacggagagaaggcgctggagtcttgcgaggcgcaggact

SEQ ID NO: 86 - DNA, 95 bp, synthetic construct
  misc_feature 1..95: note = Probe
  source 1..95: mol_type = other DNA
atgtgactggcacgggagttgatcctggttttcacctgtaagttatcgtaaaaaggagcatctaggtaggtctttgtagccaatgttacccgatt

SEQ ID NO: 87 - DNA, 95 bp, synthetic construct
  misc_feature 1..95: note = Probe
  source 1..95: mol_type = other DNA
atgtgactggcacgggagttgatcctggttttcacaatggccattcttccaggaggcacagaaattacaggccatgcacagagagaaatacccga

SEQ ID NO: 88 - DNA, 95 bp, synthetic construct
  misc_feature 1..95: note = Probe
  source 1..95: mol_type = other DNA
atgtgactggcacgggagttgatcctggttttcaccttgttcgttccttgtactgagaccctagtctgccactgaggatttggtttttgcccttc

SEQ ID NO: 89 - DNA, 95 bp, synthetic construct
  misc_feature 1..95: note = Probe
  source 1..95: mol_type = other DNA
atgtgactggcacgggagttgatcctggttttcacatcaagactcatcagtaccatcaaaagctgagatgaaacagtgtaagtttcaacagaaat

SEQ ID NO: 90 - DNA, 95 bp, synthetic construct
  misc_feature 1..95: note = Probe
  source 1..95: mol_type = other DNA
atgtgactggcacgggagttgatcctggttttcactgtgtccagctgtgaaactcagagatgtaactgctgacatcctccctattttgcatctca

SEQ ID NO: 91 - DNA, 95 bp, synthetic construct
  misc_feature 1..95: note = Probe
  source 1..95: mol_type = other DNA
atgtgactggcacgggagttgatcctggttttcacatttgaaacaattttatcatgaatgccatgaccaaagtattcttctgtatcttctttctt

SEQ ID NO: 92 - DNA, 95 bp, synthetic construct
  misc_feature 1..95: note = Probe
  source 1..95: mol_type = other DNA
atgtgactggcacgggagttgatcctggttttcactgatgggtgggctcccgaaggggcctcccgcagacttgcgaagttcccactctctgggcg

SEQ ID NO: 93 - DNA, 95 bp, synthetic construct
  misc_feature 1..95: note = Probe
  source 1..95: mol_type = other DNA
atgtgactggcacgggagttgatcctggttttcaccagggtgcgggggcatccaggctgcccaagcggaggctgggccggctgtgctggcctctt

SEQ ID NO: 94 - DNA, 95 bp, synthetic construct
  misc_feature 1..95: note = Probe
  source 1..95: mol_type = other DNA
atgtgactggcacgggagttgatcctggttttcacttttgaaatgtgggtttgttgccatgaaacgtgtttcaagcatagttttgacagataacg

SEQ ID NO: 95 - DNA, 95 bp, synthetic construct
  misc_feature 1..95: note = Probe
  source 1..95: mol_type = other DNA
atgtgactggcacgggagttgatcctggttttcactgccctaaaagtgtatgtataacatccctgatgtctgcatttgtcctttgactggtgttt

SEQ ID NO: 96 - DNA, 95 bp, synthetic construct
  misc_feature 1..95: note = Probe
  source 1..95: mol_type = other DNA
atgtgactggcacgggagttgatcctggttttcacaacccctcgaggctcagacctttggagcaggagtgtgattctggccaaccaccctctctg

SEQ ID NO: 97 - DNA, 95 bp, synthetic construct
  misc_feature 1..95: note = Probe
  source 1..95: mol_type = other DNA
atgtgactggcacgggagttgatcctggttttcaccataaatatgtgtgctagtcctgttagacccaagtgctgcccaagggcagcgccctgctc

SEQ ID NO: 98 - DNA, 95 bp, synthetic construct
  misc_feature 1..95: note = Probe
  source 1..95: mol_type = other DNA
atgtgactggcacgggagttgatcctggttttcactacttgttaattaaaaattcaagagtttttttttcttattctgaggttatctttttacca

SEQ ID NO: 99 - DNA, 95 bp, synthetic construct
  misc_feature 1..95: note = Probe
  source 1..95: mol_type = other DNA
atgtgactggcacgggagttgatcctggttttcacccaaaatctgttttccaataaattctcagatccaggaagaggaaaggaaaaacatcaaaa

SEQ ID NO: 100 - DNA, 95 bp, synthetic construct
  misc_feature 1..95: note = Probe
  source 1..95: mol_type = other DNA
atgtgactggcacgggagttgatcctggttttcacatactccatctcccgtaaaaatagtgagacttgagtaatgtttgatgtcacttgtctttc

SEQ ID NO: 101 - DNA, 95 bp, synthetic construct
  misc_feature 1..95: note = Probe
  source 1..95: mol_type = other DNA
atgtgactggcacgggagttgatcctggttttcaccagtcaccactatattattctaggtatcccagaaaagttaaagtcaaatctgaaacacat

SEQ ID NO: 102 - DNA, 95 bp, synthetic construct
  misc_feature 1..95: note = Probe
  source 1..95: mol_type = other DNA
atgtgactggcacgggagttgatcctggttttcaccgccccgcgtccgacccgcggatcccgcggcgtccggcccgggtggtctggatcgcggag

SEQ ID NO: 103 - DNA, 95 bp, synthetic construct
  misc_feature 1..95: note = Probe
  source 1..95: mol_type = other DNA
atgtgactggcacgggagttgatcctggttttcacccatacgggcagcacgacgcgcggactgcgattgcagaagatgacctgggagggctcgcg

SEQ ID NO: 104 - DNA, 95 bp, synthetic construct
  misc_feature 1..95: note = Probe
  source 1..95: mol_type = other DNA
atgtgactggcacgggagttgatcctggttttcactagaggggcttcagaccgtgctatcgtccctgctgggtcgggcctaagcgccgggcccgt

SEQ ID NO: 105 - DNA, 95 bp, synthetic construct
  misc_feature 1..95: note = Probe
  source 1..95: mol_type = other DNA
atgtgactggcacgggagttgatcctggttttcacggcgccgaggaggagatggaggccgggcggccgcggcccgtgctgcgctcggtgaactcg

SEQ ID NO: 106 - DNA, 95 bp, synthetic construct
  misc_feature 1..95: note = Probe
  source 1..95: mol_type = other DNA
atgtgactggcacgggagttgatcctggttttcacggtgtgggccaccgtgcccagccaccggtgtggctctttaacaacctttgcttgtcccga

SEQ ID NO: 107 - DNA, 95 bp, synthetic construct
  misc_feature 1..95: note = Probe
  source 1..95: mol_type = other DNA
atgtgactggcacgggagttgatcctggttttcacaagtggtctatcctgtacttaccacaacaaccttatctttttaaaaagtaaaacgtcagt

SEQ ID NO: 108 - DNA, 95 bp, synthetic construct; identical to SEQ ID NO: 88
  misc_feature 1..95: note = Probe
  source 1..95: mol_type = other DNA

SEQ ID NO: 109 - DNA, 95 bp, synthetic construct; identical to SEQ ID NO: 89
  misc_feature 1..95: note = Probe
  source 1..95: mol_type = other DNA

SEQ ID NO: 110 - DNA, 75 bp, synthetic construct
  misc_feature 1..75: note = Probe
  source 1..75: mol_type = other DNA
atgtgactggcacgggagttgatcctggttttcacacctactggatgtgcctgactgtttccccttcttcttccc

SEQ ID NO: 111 - DNA, 75 bp, synthetic construct
  misc_feature 1..75: note = Probe
  source 1..75: mol_type = other DNA
atgtgactggcacgggagttgatcctggttttcacgggaaaaaaaagatgggtctgtgtgggagggcaggtactt

SEQ ID NO: 112 - DNA, 75 bp, synthetic construct
  misc_feature 1..75: note = Probe
  source 1..75: mol_type = other DNA
atgtgactggcacgggagttgatcctggttttcacttaataagattccctggtctcgtttgtctacctgttaatg

SEQ ID NO: 113 - DNA, 75 bp, synthetic construct
  misc_feature 1..75: note = Probe
  source 1..75: mol_type = other DNA
atgtgactggcacgggagttgatcctggttttcacccccaccccttgttattgccacaaaatcctgaggatgatc

SEQ ID NO: 114 - DNA, 75 bp, synthetic construct
  misc_feature 1..75: note = Probe
  source 1..75: mol_type = other DNA
atgtgactggcacgggagttgatcctggttttcacgctgagcaggaggtggcaggtaccccagactgggaggtaa

SEQ ID NO: 115 - DNA, 75 bp, synthetic construct
  misc_feature 1..75: note = Probe
  source 1..75: mol_type = other DNA
atgtgactggcacgggagttgatcctggttttcacggcccagtctgttcacacatggctgctgcctctcagctct

SEQ ID NO: 116 - DNA, 75 bp, synthetic construct
  misc_feature 1..75: note = Probe
  source 1..75: mol_type = other DNA
atgtgactggcacgggagttgatcctggttttcacgaaagtcatttgtcaaggccttcagttggcagacgtgctc

SEQ ID NO: 117 - DNA, 75 bp, synthetic construct
  misc_feature 1..75: note = Probe
  source 1..75: mol_type = other DNA
atgtgactggcacgggagttgatcctggttttcacaatctgtggaaacgctgccacacaatcttagcacacaaga

SEQ ID NO: 118 - DNA, 75 bp, synthetic construct
  misc_feature 1..75: note = Probe
  source 1..75: mol_type = other DNA
atgtgactggcacgggagttgatcctggttttcactgcttgcaaaacaacagaatcttctctccatgaaatcatg

SEQ ID NO: 119 - DNA, 75 bp, synthetic construct
  misc_feature 1..75: note = Probe
  source 1..75: mol_type = other DNA
atgtgactggcacgggagttgatcctggttttcacattttctcacaaaggaaaccaagataaaaggtttaaatgg

SEQ ID NO: 120 - DNA, 75 bp, synthetic construct
  misc_feature 1..75: note = Probe
  source 1..75: mol_type = other DNA
atgtgactggcacgggagttgatcctggttttcactgctttctgccaaaattaatgtgctgaacttaaacttacc

SEQ ID NO: 121 - DNA, 75 bp, synthetic construct
  misc_feature 1..75: note = Probe
  source 1..75: mol_type = other DNA
atgtgactggcacgggagttgatcctggttttcacccaatgcaacagactttaaagaagttgtgttttacaatgc

SEQ ID NO: 122 - DNA, 75 bp, synthetic construct
  misc_feature 1..75: note = Probe
  source 1..75: mol_type = other DNA
atgtgactggcacgggagttgatcctggttttcacattttgcagaaaacagatctgtatttatttcagtgttact

SEQ ID NO: 123 - DNA, 75 bp, synthetic construct
  misc_feature 1..75: note = Probe
  source 1..75: mol_type = other DNA
atgtgactggcacgggagttgatcctggttttcactgtgttactaatgactgtgctataacttttttttctttcc

SEQ ID NO: 124 - DNA, 75 bp, synthetic construct
  misc_feature 1..75: note = Probe
  source 1..75: mol_type = other DNA
atgtgactggcacgggagttgatcctggttttcactgcgccaggtttccgcaccaagacccctttaactcaagac

SEQ ID NO: 125 - DNA, 75 bp, synthetic construct
  misc_feature 1..75: note = Probe
  source 1..75: mol_type = other DNA
atgtgactggcacgggagttgatcctggttttcacggggtgggcagcagctcgaatttcttccagatatcctcgc

SEQ ID NO: 126 - DNA, 75 bp, synthetic construct
  misc_feature 1..75: note = Probe
  source 1..75: mol_type = other DNA
atgtgactggcacgggagttgatcctggttttcaccatggtgaaccagagtttcatctgcgacccggacgacgag

SEQ ID NO: 127 - DNA, 75 bp, synthetic construct
  misc_feature 1..75: note = Probe
  source 1..75: mol_type = other DNA
atgtgactggcacgggagttgatcctggttttcacgacggagagaaggcgctggagtcttgcgaggcgcaggact

SEQ ID NO: 128 - DNA, 75 bp, synthetic construct
  misc_feature 1..75: note = Probe
  source 1..75: mol_type = other DNA
atgtgactggcacgggagttgatcctggttttcacgagcatctaggtaggtctttgtagccaatgttacccgatt

SEQ ID NO: 129 - DNA, 75 bp, synthetic construct
  misc_feature 1..75: note = Probe
  source 1..75: mol_type = other DNA
atgtgactggcacgggagttgatcctggttttcacgcacagaaattacaggccatgcacagagagaaatacccga

SEQ ID NO: 130 - DNA, 75 bp, synthetic construct
  misc_feature 1..75: note = Probe
  source 1..75: mol_type = other DNA
atgtgactggcacgggagttgatcctggttttcacagaccctagtctgccactgaggatttggtttttgcccttc

SEQ ID NO: 131 - DNA, 75 bp, synthetic construct
  misc_feature 1..75: note = Probe
  source 1..75: mol_type = other DNA
atgtgactggcacgggagttgatcctggttttcactcaaaagctgagatgaaacagtgtaagtttcaacagaaat

SEQ ID NO: 132 - DNA, 75 bp, synthetic construct
  misc_feature 1..75: note = Probe
  source 1..75: mol_type = other DNA
atgtgactggcacgggagttgatcctggttttcacagagatgtaactgctgacatcctccctattttgcatctca

SEQ ID NO: 133 - DNA, 75 bp, synthetic construct
  misc_feature 1..75: note = Probe
  source 1..75: mol_type = other DNA
atgtgactggcacgggagttgatcctggttttcacgaatgccatgaccaaagtattcttctgtatcttctttctt

SEQ ID NO: 134 - DNA, 75 bp, synthetic construct
  misc_feature 1..75: note = Probe
  source 1..75: mol_type = other DNA
atgtgactggcacgggagttgatcctggttttcacgggcctcccgcagacttgcgaagttcccactctctgggcg

SEQ ID NO: 135 - DNA, 75 bp, synthetic construct
  misc_feature 1..75: note = Probe
  source 1..75: mol_type = other DNA
atgtgactggcacgggagttgatcctggttttcacgctgcccaagcggaggctgggccggctgtgctggcctctt

SEQ ID NO: 136 - DNA, 75 bp, synthetic construct
  misc_feature 1..75: note = Probe
  source 1..75: mol_type = other DNA
atgtgactggcacgggagttgatcctggttttcacgccatgaaacgtgtttcaagcatagttttgacagataacg

SEQ ID NO: 137 - DNA, 75 bp, synthetic construct
  misc_feature 1..75: note = Probe
  source 1..75: mol_type = other DNA
atgtgactggcacgggagttgatcctggttttcacaacatccctgatgtctgcatttgtcctttgactggtgttt

SEQ ID NO: 138 - DNA, 75 bp, synthetic construct
  misc_feature 1..75: note = Probe
  source 1..75: mol_type = other DNA
atgtgactggcacgggagttgatcctggttttcactttggagcaggagtgtgattctggccaaccaccctctctg

SEQ ID NO: 139 - DNA, 75 bp, synthetic construct
  misc_feature 1..75: note = Probe
  source 1..75: mol_type = other DNA
atgtgactggcacgggagttgatcctggttttcacctgttagacccaagtgctgcccaagggcagcgccctgctc

SEQ ID NO: 140 - DNA, 75 bp, synthetic construct
  misc_feature 1..75: note = Probe
  source 1..75: mol_type = other DNA
atgtgactggcacgggagttgatcctggttttcacaagagtttttttttcttattctgaggttatctttttacca

SEQ ID NO: 141 - DNA, 75 bp, synthetic construct
  misc_feature 1..75: note = Probe
  source 1..75: mol_type = other DNA
atgtgactggcacgggagttgatcctggttttcacaattctcagatccaggaagaggaaaggaaaaacatcaaaa

SEQ ID NO: 142 - DNA, 75 bp, synthetic construct
  misc_feature 1..75: note = Probe
  source 1..75: mol_type = other DNA
atgtgactggcacgggagttgatcctggttttcacatagtgagacttgagtaatgtttgatgtcacttgtctttc

SEQ ID NO: 143 - DNA, 75 bp, synthetic construct
  misc_feature 1..75: note = Probe
  source 1..75: mol_type = other DNA
atgtgactggcacgggagttgatcctggttttcactaggtatcccagaaaagttaaagtcaaatctgaaacacat

SEQ ID NO: 144 - DNA, 75 bp, synthetic construct
  misc_feature 1..75: note = Probe
  source 1..75: mol_type = other DNA
atgtgactggcacgggagttgatcctggttttcacgatcccgcggcgtccggcccgggtggtctggatcgcggag

SEQ ID NO: 145 - DNA, 75 bp, synthetic construct
  misc_feature 1..75: note = Probe
  source 1..75: mol_type = other DNA
atgtgactggcacgggagttgatcctggttttcacgcggactgcgattgcagaagatgacctgggagggctcgcg

SEQ ID NO: 146 - DNA, 75 bp, synthetic construct
  misc_feature 1..75: note = Probe
  source 1..75: mol_type = other DNA
atgtgactggcacgggagttgatcctggttttcacctatcgtccctgctgggtcgggcctaagcgccgggcccgt

SEQ ID NO: 147 - DNA, 75 bp, synthetic construct
  misc_feature 1..75: note = Probe
  source 1..75: mol_type = other DNA
atgtgactggcacgggagttgatcctggttttcacggccgggcggccgcggcccgtgctgcgctcggtgaactcg

SEQ ID NO: 148 - DNA, 75 bp, synthetic construct
  misc_feature 1..75: note = Probe
  source 1..75: mol_type = other DNA
atgtgactggcacgggagttgatcctggttttcacgccaccggtgtggctctttaacaacctttgcttgtcccga

SEQ ID NO: 149 - DNA, 75 bp, synthetic construct
  misc_feature 1..75: note = Probe
  source 1..75: mol_type = other DNA
atgtgactggcacgggagttgatcctggttttcacaccacaacaaccttatctttttaaaaagtaaaacgtcagt

SEQ ID NO: 150 - DNA, 75 bp, synthetic construct; identical to SEQ ID NO: 130
  misc_feature 1..75: note = Probe
  source 1..75: mol_type = other DNA

SEQ ID NO: 151 - DNA, 75 bp, synthetic construct; identical to SEQ ID NO: 131
  misc_feature 1..75: note = Probe
  source 1..75: mol_type = other DNA

SEQ ID NO: 152 - DNA, 58 bp, synthetic construct
  misc_feature 1..58: note = ACA2_FLFP primer
  source 1..58: mol_type = other DNA
aatgatacggcgaccaccgagatctacacgtcatgcaggaccagagaattcgaataca

SEQ ID NO: 153 - DNA, 57 bp, synthetic construct
  misc_feature 1..57: note = CAC3_FLRP primer
  source 1..57: mol_type = other DNA
caagcagaagacggcatacgagatgtgactggcacgggagttgatcctggttttcac

SEQ ID NO: 154 - DNA, 75 bp, synthetic construct
  misc_feature 1..75: note = Probe
  source 1..75: mol_type = other DNA
atgtgactggcacgggagttgatcctggttttcaccgaatgagggtgatgtttttccgcggcacctccttcaggt

SEQ ID NO: 155 - DNA, 75 bp, synthetic construct
  misc_feature 1..75: note = Probe
  source 1..75: mol_type = other DNA
atgtgactggcacgggagttgatcctggttttcacgttgtagtcggtcatgatggtcgaggtgcggagcttgctc

SEQ ID NO: 156 - DNA, 75 bp, synthetic construct
  misc_feature 1..75: note = Probe
  source 1..75: mol_type = other DNA
atgtgactggcacgggagttgatcctggttttcacgcagctcctggtgcttccggcggtacactgcaggtgggtg

SEQ ID NO: 157 - DNA, 75 bp, synthetic construct
  misc_feature 1..75: note = Probe
  source 1..75: mol_type = other DNA
atgtgactggcacgggagttgatcctggttttcacctacacaggccacttcctacaggaagcctccctggatctc

SEQ ID NO: 158 - DNA, 75 bp, synthetic construct
  misc_feature 1..75: note = Probe
  source 1..75: mol_type = other DNA
atgtgactggcacgggagttgatcctggttttcacgaaatactaataaaatgattaaagaaggtgtgtctttaat

SEQ ID NO: 159 - DNA, 75 bp, synthetic construct
  misc_feature 1..75: note = Probe
  source 1..75: mol_type = other DNA
atgtgactggcacgggagttgatcctggttttcactatatggaaaataattatttgtattatatagggcagagtc

SEQ ID NO: 160 - DNA, 75 bp, synthetic construct
  misc_feature 1..75: note = Probe
  source 1..75: mol_type = other DNA
atgtgactggcacgggagttgatcctggttttcacattagacccaatatggtctgcagattttattagaagaaat

SEQ ID NO: 161 - DNA, 75 bp, synthetic construct
  misc_feature 1..75: note = Probe
  source 1..75: mol_type = other DNA
atgtgactggcacgggagttgatcctggttttcacgtgaaccagcagactgtgttgcaagtataaccccacgtga

SEQ ID NO: 162 - DNA, 75 bp, synthetic construct
  misc_feature 1..75: note = Probe
  source 1..75: mol_type = other DNA
atgtgactggcacgggagttgatcctggttttcacgccatggagcctaaggaagtttcagcaaggccctaagggg

SEQ ID NO: 163 - DNA, 75 bp, synthetic construct
  misc_feature 1..75: note = Probe
  source 1..75: mol_type = other DNA
atgtgactggcacgggagttgatcctggttttcaccccaggaattggcctgccttagtatttctgctgtgctcag

SEQ ID NO: 164 - DNA, 75 bp, synthetic construct
  misc_feature 1..75: note = Probe
  source 1..75: mol_type = other DNA
atgtgactggcacgggagttgatcctggttttcactttgagggtgcagctgggatcttggtcagttgtgtttcct

SEQ ID NO: 165 - DNA, 75 bp, synthetic construct
  misc_feature 1..75: note = Probe
  source 1..75: mol_type = other DNA
atgtgactggcacgggagttgatcctggttttcaccacatcatgaaaagatctctgaattggtgtctggggatct

SEQ ID NO: 166 - DNA, 75 bp, synthetic construct
  misc_feature 1..75: note = Probe
  source 1..75: mol_type = other DNA
atgtgactggcacgggagttgatcctggttttcactgaggaccaggtcacaggacctctttggactgcagtttcc

SEQ ID NO: 167 - DNA, 75 bp, synthetic construct
  misc_feature 1..75: note = Probe
  source 1..75: mol_type = other DNA
atgtgactggcacgggagttgatcctggttttcactaaccactgccactccccaccctctagggttgtcaatgaa

SEQ ID NO: 168 - DNA, 75 bp, synthetic construct
  misc_feature 1..75: note = Probe
  source 1..75: mol_type = other DNA
atgtgactggcacgggagttgatcctggttttcacgagctctaccaatgtgagtgaccattatcactcctacatg

SEQ ID NO: 169 - DNA, 75 bp, synthetic construct
  misc_feature 1..75: note = Probe
  source 1..75: mol_type = other DNA
atgtgactggcacgggagttgatcctggttttcacaaaattgtgattcagtgggtagattctgtgtgtaaagccc

SEQ ID NO: 170 - DNA, 75 bp, synthetic construct
  misc_feature 1..75: note = Probe
  source 1..75: mol_type = other DNA
atgtgactggcacgggagttgatcctggttttcactatgtgctcagttccctcctctatgcaatggaccgaccgt

SEQ ID NO: 171 - DNA, 75 bp, synthetic construct
  misc_feature 1..75: note = Probe
  source 1..75: mol_type = other DNA
atgtgactggcacgggagttgatcctggttttcacgtgtaaattgccgagcacgtagtaaccatgcaacaagtgt

SEQ ID NO: 172 - DNA, 75 bp, synthetic construct
  misc_feature 1..75: note = Probe
  source 1..75: mol_type = other DNA
atgtgactggcacgggagttgatcctggttttcactggggacacagtgtgtgctgccatctcccttctaccggca

SEQ ID NO: 173 - DNA, 75 bp, synthetic construct
  misc_feature 1..75: note = Probe
  source 1..75: mol_type = other DNA
atgtgactggcacgggagttgatcctggttttcacaagagcctttccctctgcccttttcaagcctctgcccatc

SEQ ID NO: 174 - DNA, 75 bp, synthetic construct
  misc_feature 1..75: note = Probe
  source 1..75: mol_type = other DNA
atgtgactggcacgggagttgatcctggttttcacgaccacactgagttctctgtgacctgcaggtcagctcacc

SEQ ID NO: 175 - DNA, 75 bp, synthetic construct
  misc_feature 1..75: note = Probe
  source 1..75: mol_type = other DNA
atgtgactggcacgggagttgatcctggttttcactttcctatctctctgcctggagggtggtggagggctggtt

SEQ ID NO: 176 - DNA, 75 bp, synthetic construct
  misc_feature 1..75: note = Probe
  source 1..75: mol_type = other DNA
atgtgactggcacgggagttgatcctggttttcacaaacaggagctgcgccggtggaagcatgtgggagctagaa

SEQ ID NO: 177 - DNA, 75 bp, synthetic construct
  misc_feature 1..75: note = Probe
  source 1..75: mol_type = other DNA
atgtgactggcacgggagttgatcctggttttcacggacactgaaggagctccccaccccctgatcagccaggag

SEQ ID NO: 178 - DNA, 75 bp, synthetic construct
  misc_feature 1..75: note = Probe
  source 1..75: mol_type = other DNA
atgtgactggcacgggagttgatcctggttttcacgggaactgcagctgctctggtggggggaaggttgggagct

SEQ ID NO: 179 - DNA, 75 bp, synthetic construct
  misc_feature 1..75: note = Probe
  source 1..75: mol_type = other DNA
atgtgactggcacgggagttgatcctggttttcacacccaattccagggactagcataacgaagtgacaccttgg

SEQ ID NO: 180 - DNA, 75 bp, synthetic construct
  misc_feature 1..75: note = Probe
  source 1..75: mol_type = other DNA
atgtgactggcacgggagttgatcctggttttcaccctgcccccttgggagtccctggggctctgtgcactcacc

SEQ ID NO: 181 - DNA, 75 bp, synthetic construct
  misc_feature 1..75: note = Probe
  source 1..75: mol_type = other DNA
atgtgactggcacgggagttgatcctggttttcacggaagcacccccggtattaaaacgaacggggcggaaagaa

SEQ ID NO: 182 - DNA, 75 bp, synthetic construct
  misc_feature 1..75: note = Probe
  source 1..75: mol_type = other DNA
atgtgactggcacgggagttgatcctggttttcacctaacaaaggggacgcgacccggggtccagtgccccaggg

SEQ ID NO: 183 - DNA, 75 bp, synthetic construct
  misc_feature 1..75: note = Probe
  source 1..75: mol_type = other DNA
atgtgactggcacgggagttgatcctggttttcaccctggggggactgggtggcctcacccccaacccggtcatc

SEQ ID NO: 184 - DNA, 75 bp, synthetic construct
  misc_feature 1..75: note = Probe
  source 1..75: mol_type = other DNA
atgtgactggcacgggagttgatcctggttttcaccgcgctccagcttctcgcgggcggagaagccgctccacat

SEQ ID NO: 185 - DNA, 75 bp, synthetic construct
  misc_feature 1..75: note = Probe
  source 1..75: mol_type = other DNA
atgtgactggcacgggagttgatcctggttttcaccccacccggccgccgagtgcgtggatcccgccgtggtctt

SEQ ID NO: 186 - DNA, 75 bp, synthetic construct
  misc_feature 1..75: note = Probe
  source 1..75: mol_type = other DNA
atgtgactggcacgggagttgatcctggttttcacgggcacgggcgctggctcgcgcttgttcacgggaaagggg

SEQ ID NO: 187 - DNA, 75 bp, synthetic construct
  misc_feature 1..75: note = Probe
  source 1..75: mol_type = other DNA
atgtgactggcacgggagttgatcctggttttcacaacatggatatatatgtgaatttcattcaaatggttctca

SEQ ID NO: 188 - DNA, 75 bp, synthetic construct
  misc_feature 1..75: note = Probe
  source 1..75: mol_type = other DNA
atgtgactggcacgggagttgatcctggttttcactaaaccaacattcttaatgtcaacacaatgtttgtttaaa

SEQ ID NO: 189 - DNA, 75 bp, synthetic construct
  misc_feature 1..75: note = Probe
  source 1..75: mol_type = other DNA
atgtgactggcacgggagttgatcctggttttcacccctacgtggagagtgaggatgcacccccacagaagaaga

SEQ ID NO: 190 - DNA, 75 bp, synthetic construct
  misc_feature 1..75: note = Probe
  source 1..75: mol_type = other DNA
atgtgactggcacgggagttgatcctggttttcacatgacactcttgagcggacgtggggacgcctcgctcttta

SEQ ID NO: 191 - DNA, 75 bp, synthetic construct
  misc_feature 1..75: note = Probe
  source 1..75: mol_type = other DNA
atgtgactggcacgggagttgatcctggttttcactctcacgctcagggaccacgtgccggagttggtaaagaat

SEQ ID NO: 192 - DNA, 75 bp, synthetic construct
  misc_feature 1..75: note = Probe
  source 1..75: mol_type = other DNA
atgtgactggcacgggagttgatcctggttttcaccagtggcctttttcaaaatgaccaccttggcggccttctc

SEQ ID NO: 193 - DNA, 75 bp, synthetic construct
  misc_feature 1..75: note = Probe
  source 1..75: mol_type = other DNA
atgtgactggcacgggagttgatcctggttttcacgctagggggctggggttggggtgggggtggtgggcctgcc

SEQ ID NO: 194 - DNA, 75 bp, synthetic construct
  misc_feature 1..75: note = Probe
  source 1..75: mol_type = other DNA
atgtgactggcacgggagttgatcctggttttcaccagtttccataggtctgaaaatgtttcctgactcagaggg

SEQ ID NO: 195 - DNA, 75 bp, synthetic construct
  misc_feature 1..75: note = Probe
  source 1..75: mol_type = other DNA
atgtgactggcacgggagttgatcctggttttcacctgccatggaggagccgcagtcagatcctagcgtcgagcc

SEQ ID NO: 196 - DNA, 75 bp, synthetic construct
  misc_feature 1..75: note = Probe
  source 1..75: mol_type = other DNA
atgtgactggcacgggagttgatcctggttttcactcatgctggatccccacttttcctcttgcagcagccagac

SEQ ID NO: 197 - DNA, 75 bp, synthetic construct
  misc_feature 1..75: note = Probe
  source 1..75: mol_type = other DNA
atgtgactggcacgggagttgatcctggttttcacagccccccagccctccaggtccccagccctccaggtcccc

SEQ ID NO: 198 - DNA, 75 bp, synthetic construct
  misc_feature 1..75: note = Probe
  source 1..75: mol_type = other DNA
atgtgactggcacgggagttgatcctggttttcacgcagagacctgtgggaagcgaaaattccatgggactgact

SEQ ID NO: 199 - DNA, 75 bp, synthetic construct
  misc_feature 1..75: note = Probe
  source 1..75: mol_type = other DNA
atgtgactggcacgggagttgatcctggttttcacgcagggggatacggccaggcattgaagtctcatggaagcc

SEQ ID NO: 200 - DNA, 75 bp, synthetic construct
  misc_feature 1..75: note = Probe
  source 1..75: mol_type = other DNA
atgtgactggcacgggagttgatcctggttttcacccgtgcaagtcacagacttggctgtcccagaatgcaagaa

SEQ ID NO: 201 - DNA, 75 bp, synthetic construct
  misc_feature 1..75: note = Probe
  source 1..75: mol_type = other DNA
atgtgactggcacgggagttgatcctggttttcacccagaaaacctaccagggcagctacggtttccgtctgggc

SEQ ID NO: 202 - DNA, 75 bp, synthetic construct
  misc_feature 1..75: note = Probe
  source 1..75: mol_type = other DNA
atgtgactggcacgggagttgatcctggttttcacgaagggacagaagatgacaggggccaggagggggctggtg

SEQ ID NO: 203 - DNA, 75 bp, synthetic construct
  misc_feature 1..75: note = Probe
  source 1..75: mol_type = other DNA
atgtgactggcacgggagttgatcctggttttcacgtggcccctgcaccagcagctcctacaccggcggcccctg

SEQ ID NO: 204 - DNA, 75 bp, synthetic construct
  misc_feature 1..75: note = Probe
  source 1..75: mol_type = other DNA
atgtgactggcacgggagttgatcctggttttcacggggggagcagcctctggcattctgggagcttcatctgga

SEQ ID NO: 205 - DNA, 75 bp, synthetic construct
  misc_feature 1..75: note = Probe
  source 1..75: mol_type = other DNA
atgtgactggcacgggagttgatcctggttttcacccccggacgatattgaacaatggttcactgaagacccagg

SEQ ID NO: 206 - DNA, 75 bp, synthetic construct
  misc_feature 1..75: note = Probe
  source 1..75: mol_type = other DNA
atgtgactggcacgggagttgatcctggttttcacctggggggctggggggctgaggacctggtcctctgactgc

SEQ ID NO: 207 - DNA, 75 bp, synthetic construct
  misc_feature 1..75: note = Probe
  source 1..75: mol_type = other DNA
atgtgactggcacgggagttgatcctggttttcaccctgggcaaccagccctgtcgtctctccagccccagctgc

SEQ ID NO: 208 - DNA, 75 bp, synthetic construct
  misc_feature 1..75: note = Probe
  source 1..75: mol_type = other DNA
atgtgactggcacgggagttgatcctggttttcacccatcgctatctgagcagcgctcatggtgggggcagcgcc

SEQ ID NO: 209 - DNA, 75 bp, synthetic construct
  misc_feature 1..75: note = Probe
  source 1..75: mol_type = other DNA
atgtgactggcacgggagttgatcctggttttcacgccatctacaagcagtcacagcacatgacggaggttgtga

SEQ ID NO: 210 - DNA, 75 bp, synthetic construct
  misc_feature 1..75: note = Probe
  source 1..75: mol_type = other DNA
atgtgactggcacgggagttgatcctggttttcaccatggcgcggacgcgggtgccgggcgggggtgtggaatca

SEQ ID NO: 211 - DNA, 75 bp, synthetic construct
  misc_feature 1..75: note = Probe
  source 1..75: mol_type = other DNA
atgtgactggcacgggagttgatcctggttttcactttgccaactggccaagacctgccctgtgcagctgtgggt

SEQ ID NO: 212 - DNA, 75 bp, synthetic construct
  misc_feature 1..75: note = Probe
  source 1..75: mol_type = other DNA
atgtgactggcacgggagttgatcctggttttcactgctttatctgttcacttgtgccctgactttcaactctgt

SEQ ID NO: 213 - DNA, 75 bp, synthetic construct
  misc_feature 1..75: note = Probe
  source 1..75: mol_type = other DNA
atgtgactggcacgggagttgatcctggttttcacgagggccactgacaaccacccttaacccctcctcccagag

SEQ ID NO: 214 - DNA, 75 bp, synthetic construct
  misc_feature 1..75: note = Probe
  source 1..75: mol_type = other DNA
atgtgactggcacgggagttgatcctggttttcaccctcaggcggctcatagggcaccaccacactatgtcgaaa

SEQ ID NO: 215 - DNA, 75 bp, synthetic construct
  misc_feature 1..75: note = Probe
  source 1..75: mol_type = other DNA
atgtgactggcacgggagttgatcctggttttcacaggaaatttgcgtgtggagtatttggatgacagaaacact

SEQ ID NO: 216 - DNA, 75 bp, synthetic construct
  misc_feature 1..75: note = Probe
  source 1..75: mol_type = other DNA
atgtgactggcacgggagttgatcctggttttcacccagggtccccaggcctctgattcctcactgattgctctt

SEQ ID NO: 217 - DNA, 75 bp, synthetic construct
  misc_feature 1..75: note = Probe
  source 1..75: mol_type = other DNA
atgtgactggcacgggagttgatcctggttttcacgaggcaagcagaggctggggcacagcaggccagtgtgcag

SEQ ID NO: 218 - DNA, 75 bp, synthetic construct
  misc_feature 1..75: note = Probe
  source 1..75: mol_type = other DNA
atgtgactggcacgggagttgatcctggttttcaccctggagtcttccagtgtgatgatggtgaggatgggcctc

SEQ ID NO: 219 - DNA, 75 bp, synthetic construct
  misc_feature 1..75: note = Probe
  source 1..75: mol_type = other DNA
atgtgactggcacgggagttgatcctggttttcacactacatgtgtaacagttcctgcatgggcggcatgaaccg

SEQ ID NO: 220 - DNA, 75 bp, synthetic construct
  misc_feature 1..75: note = Probe
  source 1..75: mol_type = other DNA
atgtgactggcacgggagttgatcctggttttcaccttgccacaggtctccccaaggcgcactggcctcatcttg

SEQ ID NO: 221 - DNA, 75 bp, synthetic construct
  misc_feature 1..75: note = Probe
  source 1..75: mol_type = other DNA
atgtgactggcacgggagttgatcctggttttcacctgcacccttggtctcctccaccgcttcttgtcctgcttg

SEQ ID NO: 222 - DNA, 75 bp, synthetic construct
  misc_feature 1..75: note = Probe
  source 1..75: mol_type = other DNA
atgtgactggcacgggagttgatcctggttttcaccctcgcttagtgctccctgggggcagctcgtggtgaggct

SEQ ID NO: 223 - DNA, 75 bp, synthetic construct
  misc_feature 1..75: note = Probe
  source 1..75: mol_type = other DNA
atgtgactggcacgggagttgatcctggttttcacgaccggcgcacagaggaagagaatctccgcaagaaagggg

SEQ ID NO: 224 - DNA, 75 bp, synthetic construct
  misc_feature 1..75: note = Probe
  source 1..75: mol_type = other DNA
atgtgactggcacgggagttgatcctggttttcactctcccaggacaggcacaaacacgcacctcaaagctgttc

SEQ ID NO: 225 - DNA, 75 bp, synthetic construct
  misc_feature 1..75: note = Probe
  source 1..75: mol_type = other DNA
atgtgactggcacgggagttgatcctggttttcactctcttttcctatcctgagtagtggtaatctactgggacg

SEQ ID NO: 226 - DNA, 75 bp, synthetic construct
  misc_feature 1..75: note = Probe
  source 1..75: mol_type = other DNA
atgtgactggcacgggagttgatcctggttttcacggacaggtaggacctgatttccttactgcctcttgcttct

SEQ ID NO: 227 - DNA, 75 bp, synthetic construct
  misc_feature 1..75: note = Probe
  source 1..75: mol_type = other DNA
atgtgactggcacgggagttgatcctggttttcacggcattttgagtgttagactggaaactttccacttgataa

SEQ ID NO: 228 - DNA, 75 bp, synthetic construct
  misc_feature 1..75: note = Probe
  source 1..75: mol_type = other DNA
atgtgactggcacgggagttgatcctggttttcaccctgaagggtgaaatattctccatccagtggtttcttctt

SEQ ID NO: 229 - DNA, 75 bp, synthetic construct
  misc_feature 1..75: note = Probe
  source 1..75: mol_type = other DNA
atgtgactggcacgggagttgatcctggttttcaccctagcactgcccaacaacaccagctcctctccccagcca

SEQ ID NO: 230 - DNA, 75 bp, synthetic construct
  misc_feature 1..75: note = Probe
  source 1..75: mol_type = other DNA
atgtgactggcacgggagttgatcctggttttcactgcctcagattcacttttatcacctttccttgcctctttc

SEQ ID NO: 231 - DNA, 75 bp, synthetic construct
  misc_feature 1..75: note = Probe
  source 1..75: mol_type = other DNA
atgtgactggcacgggagttgatcctggttttcacatggctttccaacctaggaaggcaggggagtagggccagg

SEQ ID NO: 232 - DNA, 75 bp, synthetic construct
  misc_feature 1..75: note = Probe
  source 1..75: mol_type = other DNA
atgtgactggcacgggagttgatcctggttttcaccctggagtgagccctgctcccccctggctccttcccagcc

SEQ ID NO: 233 - DNA, 75 bp, synthetic construct
  misc_feature 1..75: note = Probe
  source 1..75: mol_type = other DNA
atgtgactggcacgggagttgatcctggttttcactccgagagctgaatgaggccttggaactcaaggatgccca

SEQ ID NO: 234 - DNA, 75 bp, synthetic construct
  misc_feature 1..75: note = Probe
  source 1..75: mol_type = other DNA
atgtgactggcacgggagttgatcctggttttcaccatcttttaactcaggtactgtgtatatacttacttctcc

SEQ ID NO: 235 - DNA, 75 bp, synthetic construct
  misc_feature 1..75: note = Probe
  source 1..75: mol_type = other DNA
atgtgactggcacgggagttgatcctggttttcacggcaggggagggagagatgggggtgggaggctgtcagtgg

SEQ ID NO: 236 - DNA, 75 bp, synthetic construct
  misc_feature 1..75: note = Probe
  source 1..75: mol_type = other DNA
atgtgactggcacgggagttgatcctggttttcacgtcagtctgagtcaggcccttctgtcttgaacatgagttt

SEQ ID NO: 237 - DNA, 75 bp, synthetic construct
  misc_feature 1..75: note = Probe
  source 1..75: mol_type = other DNA
atgtgactggcacgggagttgatcctggttttcaccctgaagtccaaaaagggtcagtctacctcccgccataaa

SEQ ID NO: 238 - DNA, 75 bp, synthetic construct
  misc_feature 1..75: note = Probe
  source 1..75: mol_type = other DNA
atgtgactggcacgggagttgatcctggttttcacggcacagaccctctcactcatgtgatgtcatctctcctcc

SEQ ID NO: 239 - DNA, 75 bp, synthetic construct
  misc_feature 1..75: note = Probe
  source 1..75: mol_type = other DNA
atgtgactggcacgggagttgatcctggttttcaccaggggcttatgtgtctccttgatgacctgcggcgacgtc

SEQ ID NO: 240 - DNA, 75 bp, synthetic construct
  misc_feature 1..75: note = Probe
  source 1..75: mol_type = other DNA
atgtgactggcacgggagttgatcctggttttcacccatcatctcctcccttccccttctgcccaggctgttgca

SEQ ID NO: 241 - DNA, 75 bp, synthetic construct
  misc_feature 1..75: note = Probe
  source 1..75: mol_type = other DNA
atgtgactggcacgggagttgatcctggttttcacaattctggcttctccctgctcacactttcttccattgcat

SEQ ID NO: 242 - DNA, 75 bp, synthetic construct
  misc_feature 1..75: note = Probe
  source 1..75: mol_type = other DNA
atgtgactggcacgggagttgatcctggttttcacgtcagctcgtgttggcaacataccatcttcaacctctgca

SEQ ID NO: 243 - DNA, 75 bp, synthetic construct
  misc_feature 1..75: note = Probe
  source 1..75: mol_type = other DNA
atgtgactggcacgggagttgatcctggttttcactaatttcttggcccctcttcggtaaccctgagccaaatgt

SEQ ID NO: 244 - DNA, 75 bp, synthetic construct
  misc_feature 1..75: note = Probe
  source 1..75: mol_type = other DNA
atgtgactggcacgggagttgatcctggttttcacggtgaaataaaggaagatactagttttgctgaaaatgaca

SEQ ID NO: 245 - DNA, 75 bp, synthetic construct
  misc_feature 1..75: note = Probe
  source 1..75: mol_type = other DNA
atgtgactggcacgggagttgatcctggttttcacactcatttgtatctgaagtggaaccaaatgatactgatcc

SEQ ID NO: 246 - DNA, 75 bp, synthetic construct
  misc_feature 1..75: note = Probe
  source 1..75: mol_type = other DNA
atgtgactggcacgggagttgatcctggttttcacagttgagaccattcacaggccaaagacggtacaacttcct

SEQ ID NO: 247 - DNA, 75 bp, synthetic construct
  misc_feature 1..75: note = Probe
  source 1..75: mol_type = other DNA
atgtgactggcacgggagttgatcctggttttcacgaaaatgaatgctctgagctttggaagctctcagggtaca

SEQ ID NO: 248 - DNA, 75 bp, synthetic construct
  misc_feature 1..75: note = Probe
  source 1..75: mol_type = other DNA
atgtgactggcacgggagttgatcctggttttcacgggccatcgcgatgtcgcacggtacctgcgcgcggctgcg

SEQ ID NO: 249 - DNA, 75 bp, synthetic construct
  misc_feature 1..75: note = Probe
  source 1..75: mol_type = other DNA
atgtgactggcacgggagttgatcctggttttcacccccatccagcttcaaaagctcttcgaatcattgatgtgc

SEQ ID NO: 250 - DNA, 75 bp, synthetic construct
  misc_feature 1..75: note = Probe
  source 1..75: mol_type = other DNA
atgtgactggcacgggagttgatcctggttttcactgccaagcctgaactacccctcttttacactcctattgat

SEQ ID NO: 251 - DNA, 75 bp, synthetic construct
  misc_feature 1..75: note = Probe
  source 1..75: mol_type = other DNA
atgtgactggcacgggagttgatcctggttttcacccaccctgactgtgctctgtccccccagggctggacatcc

SEQ ID NO: 252 - DNA, 75 bp, synthetic construct
  misc_feature 1..75: note = Probe
  source 1..75: mol_type = other DNA
atgtgactggcacgggagttgatcctggttttcacagtcaggagtgggatgatcttataaaactcgtagaaagag

SEQ ID NO: 253 - DNA, 75 bp, synthetic construct
  misc_feature 1..75: note = Probe
  source 1..75: mol_type = other DNA
atgtgactggcacgggagttgatcctggttttcaccttcggggagacaacgacggcggtggcgggagcttctcca

SEQ ID NO: 254 - DNA, 75 bp, synthetic construct
  misc_feature 1..75: note = Probe
  source 1..75: mol_type = other DNA
atgtgactggcacgggagttgatcctggttttcaccatacagtcctggatgatgatgtttttgatgaaggtctcg

SEQ ID NO: 255 - DNA, 75 bp, synthetic construct
  misc_feature 1..75: note = Probe
  source 1..75: mol_type = other DNA
atgtgactggcacgggagttgatcctggttttcacttttactgttcttcctcagacattcaaacgtgttttgatc

SEQ ID NO: 256 - DNA, 75 bp, synthetic construct
  misc_feature 1..75: note = Probe
  source 1..75: mol_type = other DNA
atgtgactggcacgggagttgatcctggttttcacgtggaagcatactgcaaaatatttgttttcagtctctgca

SEQ ID NO: 257 - DNA, 75 bp, synthetic construct
  misc_feature 1..75: note = Probe
  source 1..75: mol_type = other DNA
atgtgactggcacgggagttgatcctggttttcacacgtacccctctcagcccctcctcttggactccagccatg

SEQ ID NO: 258 - DNA, 75 bp, synthetic construct
  misc_feature 1..75: note = Probe
  source 1..75: mol_type = other DNA
atgtgactggcacgggagttgatcctggttttcacgtggcgtaagcgcggcacgcggcgcagtggtccccgtcct

SEQ ID NO: 259 - DNA, 21 bp, synthetic construct
  misc_feature 1..21: note = Adaptor
  misc_feature 1..5: note = n is a, c, g, or t
  source 1..21: mol_type = other DNA
nnnnnaagatcttagtggcac

SEQ ID NO: 260 - DNA, 21 bp, synthetic construct
  misc_feature 1..21: note = Adaptor
  misc_feature 1..5: note = n is a, c, g, or t
  source 1..21: mol_type = other DNA
nnnnncgacagaactattgcc

SEQ ID NO: 261 - DNA, 21 bp, synthetic construct
  misc_feature 1..21: note = Adaptor
  misc_feature 1..21: note = n is a, c, g, or t
  misc_feature 1..5: note = n is a, c, g, or t
  source 1..21: mol_type = other DNA
nnnnnactatcttagtggcac

SEQ ID NO: 262 - DNA, 21 bp, synthetic construct
  misc_feature 1..21: note = Adaptor
  misc_feature 1..5: note = n is a, c, g, or t
  source 1..21: mol_type = other DNA
nnnnnctccagaactattgcc

SEQ ID NO: 263 - DNA, 21 bp, synthetic construct
  misc_feature 1..21: note = Adaptor
  misc_feature 1..5: note = n is a, c, g, or t
  source 1..21: mol_type = other DNA
nnnnnagcatcttagtggcac

SEQ ID NO: 264 - DNA, 21 bp, synthetic construct
  misc_feature 1..21: note = Adaptor
  misc_feature 1..5: note = n is a, c, g, or t
  source 1..21: mol_type = other DNA
nnnnncatcagaactattgcc

SEQ ID NO: 265 - DNA, 21 bp, synthetic construct
  misc_feature 1..21: note = Adaptor
  misc_feature 1..5: note = n is a, c, g, or t
  source 1..21: mol_type = other DNA
nnnnnataatcttagtggcac

SEQ ID NO: 266 - DNA, 21 bp, synthetic construct
  misc_feature 1..21: note = Adaptor
  misc_feature 1..5: note = n is a, c, g, or t
  source 1..21: mol_type = other DNA
nnnnnaagaaggtagaccctc

SEQ ID NO: 267 - DNA, 21 bp, synthetic construct
  misc_feature 1..21: note = Adaptor
  misc_feature 1..5: note = n is a, c, g, or t
  source 1..21: mol_type = other DNA
nnnnntttctctactcgtgac

SEQ ID NO: 268 - DNA, 21 bp, synthetic construct
  misc_feature 1..21: note = Adaptor
  misc_feature 1..5: note = n is a, c, g, or t
  source 1..21: mol_type = other DNA
nnnnnactaaggtagaccctc

SEQ ID NO: 269 - DNA, 21 bp, synthetic construct
  misc_feature 1..21: note = Adaptor
  misc_feature 1..5: note = n is a, c, g, or t
  source 1..21: mol_type = other DNA
nnnnngaagctacgagtatcc

SEQ ID NO: 270 - DNA, 21 bp, synthetic construct
  misc_feature 1..21: note = Adaptor
  misc_feature 1..5: note = n is a, c, g, or t
  source 1..21: mol_type = other DNA
nnnnnagcaaggtagaccctc

SEQ ID NO: 271 - DNA, 21 bp, synthetic construct
  misc_feature 1..21: note = Adaptor
  misc_feature 1..5: note = n is a, c, g, or t
  source 1..21: mol_type = other DNA
nnnnncattgacgtctagagc

SEQ ID NO: 272 - DNA, 21 bp, synthetic construct
  misc_feature 1..21: note = Adaptor
  misc_feature 1..5: note = n is a, c, g, or t
  source 1..21: mol_type = other DNA
nnnnntcactctactcgtgac

SEQ ID NO: 273 - DNA, 21 bp, synthetic construct
  misc_feature 1..21: note = Adaptor
  misc_feature 1..5: note = n is a, c, g, or t
  source 1..21: mol_type = other DNA
nnnnnataaaggtagaccctc

SEQ ID NO: 274 - DNA, 21 bp, synthetic construct
  misc_feature 1..21: note = Adaptor
  misc_feature 1..5: note = n is a, c, g, or t
  source 1..21: mol_type = other DNA
nnnnntacctctactcgtgac

SEQ ID NO: 275 - DNA, 20 bp, synthetic construct
  misc_feature 1..20: note = Adaptor
  misc_feature 1..5: note = n is a, c, g, or t
  source 1..20: mol_type = other DNA
nnnnnttttgtgtgtgtgtg

SEQ ID NO: 276 - DNA, 20 bp, synthetic construct
  misc_feature 1..20: note = Adaptor
  misc_feature 1..5: note = n is a, c, g, or t
  source 1..20: mol_type = other DNA
nnnnnactacacacacacac

SEQ ID NO: 277 - DNA, 20 bp, synthetic construct
  misc_feature 1..20: note = Adaptor
  misc_feature 1..5: note = n is a, c, g, or t
  source 1..20: mol_type = other DNA
nnnnnctcgtgtgtgtgtgt

SEQ ID NO: 278 - DNA, 20 bp, synthetic construct
  misc_feature 1..20: note = Adaptor
  misc_feature 1..5: note = n is a, c, g, or t
  source 1..20: mol_type = other DNA
nnnnngaacacacacacaca

SEQ ID NO: 279 - DNA, 20 bp, synthetic construct
  misc_feature 1..20: note = Adaptor
  misc_feature 1..5: note = n is a, c, g, or t
  source 1..20: mol_type = other DNA
nnnnncatgtgtgtgtgtgt

SEQ ID NO: 280 - DNA, 20 bp, synthetic construct
  misc_feature 1..20: note = Adaptor
  misc_feature 1..5: note = n is a, c, g, or t
  source 1..20: mol_type = other DNA
nnnnngtgcacacacacaca

SEQ ID NO: 281 - DNA, 20 bp, synthetic construct
  misc_feature 1..20: note = Adaptor
  misc_feature 1..5: note = n is a, c, g, or t
  source 1..20: mol_type = other DNA
nnnnnataacacacacacac

SEQ ID NO: 282 - DNA, 20 bp, synthetic construct
  misc_feature 1..20: note = Adaptor
  misc_feature 1..5: note = n is a, c, g, or t
  source 1..20: mol_type = other DNA
nnnnntactgtgtgtgtgtg

SEQ ID NO: 283 - DNA, 25 bp, synthetic construct
  misc_feature 1..25: note = Primer
  source 1..25: mol_type = other DNA
tgcaggaccagagaattcgaataca

SEQ ID NO: 284 - DNA, 58 bp, synthetic construct; identical to SEQ ID NO: 152
  misc_feature 1..58: note = Primer
  source 1..58: mol_type = other DNA

SEQ ID NO: 285 - DNA, 18 bp, synthetic construct
  misc_feature 1..18: note = Primer
  source 1..18: mol_type = other DNA
cggtggctcacgcctgta

SEQ ID NO: 286 - DNA, 18 bp, synthetic construct
  misc_feature 1..18: note = Primer
  source 1..18: mol_type = other DNA
gcctcggcctcccaaagt

SEQ ID NO: 287 - DNA, 21 bp, synthetic construct
  misc_feature 1..21: note = Primer
  source 1..21: mol_type = other DNA
gaggctgaggcaggagaatcg

SEQ ID NO: 288 - DNA, 18 bp, synthetic construct
  misc_feature 1..18: note = Primer
  source 1..18: mol_type = other DNA
gtcgcccaggctggagtg

SEQ ID NO: 289 - DNA, 25 bp, synthetic construct
  misc_feature 1..25: note = Element 1
  source 1..25: mol_type = other DNA
tgcaggaccagagaattcgaataca

SEQ ID NO: 290-554 - skipped (265 entries)

SEQ ID NO: 555 - DNA, 12 bp, synthetic construct
  misc_feature 1..12: note = Element 4
  source 1..12: mol_type = other DNA
acccacaccaaa

SEQ ID NO: 556 - DNA, 12 bp, synthetic construct
  misc_feature 1..12: note = Element 4
  source 1..12: mol_type = other DNA
caaacacaaccc

SEQ ID NO: 557 - DNA, 12 bp, synthetic construct
  misc_feature 1..12: note = Element 4
  source 1..12: mol_type = other DNA
gtgtgggttgtt

SEQ ID NO: 558 - DNA, 12 bp, synthetic construct
  misc_feature 1..12: note = Element 4
  source 1..12: mol_type = other DNA
tgtgtttggtgg

SEQ ID NO: 559 - DNA, 12 bp, synthetic construct
  misc_feature 1..12: note = Element 4
  source 1..12: mol_type = other DNA
tttggtgtgggt

SEQ ID NO: 560 - DNA, 12 bp, synthetic construct
  misc_feature 1..12: note = Element 4
  source 1..12: mol_type = other DNA
gggttgtgtttg

SEQ ID NO: 561 - DNA, 12 bp, synthetic construct
  misc_feature 1..12: note = Element 4
  source 1..12: mol_type = other DNA
aacaacccacac

SEQ ID NO: 562 - DNA, 12 bp, synthetic construct
  misc_feature 1..12: note = Element 4
  source 1..12: mol_type = other DNA
ccaccaaacaca